European Patent Application EP 4 141 023 A1, published March 1, 2023. Title: Protein variants having GLP-1 inducing activity and their use. Applicant: Ko BioLabs, Inc. The sequence listing filed with the application follows.

SEQUENCE LISTING (193 sequences)

SEQ ID NO: 1 - protein, 748 aa, Unknown
  Akkermansia muciniphila SNUG-61027 (KBL983) B2UMO7
MEKNAPFSVMNMHSFRWIRLTAFSALAAAAITSCASAATDFNQVGKQMSLLLQNFHFSRKEFSDELSTKFLETYLRKVDPNKIFFTQQDVDALKRKYGKELDDYLMSGQMMDAAQAMHALYRQRAMQRISYARDLLKKGGFTFDKDKSIERSRRKTAAWPKDEAEMQQVWKDMVEEQLLSEILRRETVARLAKEQNKPDPLANEKPAEEKLLMRYERIQRNIQETDLEDVAETLLSAVALTYDPHTDYMGARQVDRFKISMGTELTGIGALLGSEDDGSTKITGIVVGGPADKSGELKLNDRIVAIDSDNSGEMVDILFMKLDKVVDMIRGAENTQMRLKVEPADAPGQAKIITLTRSKVPLKDELAKGEIIELTGAPEGRNRIGVLSLPSFYADMEGGDRRCAKDVKKILERMNKENVDGLVIDLRSNGGGSLEEVRLMTGFFTGNGPVVQIKDTRGNVDIKSAHNRQKLFNGPIVVLINKLSASASEILAAALQDYGRAVIVGDESTFGKGSVQQPVDIGQYLPFFAARDRAGLLKVTTQKFYRVAGGSTQLKGVESDIQLPTATAAFELGEDILDYAMPYDQITPCTNYKKDSSIAAMLPVLKDASAKRVEKDRDLQIAREDIAMMKQRIKDNKLSLNKKIREQENSALEERRKSINKERKIRFAEMAKEDATKYKIYRLTLDDVNAKELPLADPEKDNEQFMHLAEDPTAELDDSPEYPSGLDPELREGINIVQDMLKLESSGK

SEQ ID NO: 2 - protein, 745 aa, Unknown
  P9-01(10-748-His)
MNMHSFRWIRLTAFSALAAAAITSCASAATDFNQVGKQMSLLLQNFHFSRKEFSDELSTKFLETYLRKVDPNKIFFTQQDVDALKRKYGKELDDYLMSGQMMDAAQAMHALYRQRAMQRISYARDLLKKGGFTFDKDKSIERSRRKTAAWPKDEAEMQQVWKDMVEEQLLSEILRRETVARLAKEQNKPDPLANEKPAEEKLLMRYERIQRNIQETDLEDVAETLLSAVALTYDPHTDYMGARQVDRFKISMGTELTGIGALLGSEDDGSTKITGIVVGGPADKSGELKLNDRIVAIDSDNSGEMVDILFMKLDKVVDMIRGAENTQMRLKVEPADAPGQAKIITLTRSKVPLKDELAKGEIIELTGAPEGRNRIGVLSLPSFYADMEGGDRRCAKDVKKILERMNKENVDGLVIDLRSNGGGSLEEVRLMTGFFTGNGPVVQIKDTRGNVDIKSAHNRQKLFNGPIVVLINKLSASASEILAAALQDYGRAVIVGDESTFGKGSVQQPVDIGQYLPFFAARDRAGLLKVTTQKFYRVAGGSTQLKGVESDIQLPTATAAFELGEDILDYAMPYDQITPCTNYKKDSSIAAMLPVLKDASAKRVEKDRDLQIAREDIAMMKQRIKDNKLSLNKKIREQENSALEERRKSINKERKIRFAEMAKEDATKYKIYRLTLDDVNAKELPLADPEKDNEQFMHLAEDPTAELDDSPEYPSGLDPELREGINIVQDMLKLESSGKHHHHHH

SEQ ID NO: 3 - DNA, 2217 bp, Unknown
  P9(10-748)
atgaacatgcactcattccgttggattagactcaccgcattctcggccctggccgcagccgccattacttcctgcgcctctgcggctacggacttcaaccaggtgggcaagcaaatgtccctgctgctccagaatttccacttctcccgcaaagaattcagcgatgaactatccactaaattcctggaaacctacctgcgcaaggtagaccccaacaaaatattcttcacccagcaggacgtagacgccctcaaaagaaaatacggtaaggagctggacgactaccttatgtccggccagatgatggatgcggcccaggccatgcacgccctttaccgccagcgcgccatgcagcgcatctcctatgcgcgggatttgctgaaaaagggaggcttcacctttgacaaagacaagtctatcgaacgttcccgccgcaaaacagccgcgtggcccaaggatgaggcggaaatgcagcaggtctggaaagacatggtggaggaacagctcctgtccgaaatcctgcgccgtgaaaccgtagcgcgcctggccaaggaacagaacaagcccgatcccctggccaatgaaaaacccgcggaggaaaaactgcttatgcgttatgaacgcattcagcgcaatattcaggaaacggatctggaagacgtagcggaaacactgctcagcgccgtagccttgacgtatgacccgcatacggattacatgggtgcgcgccaagtggaccgtttcaaaatctccatgggtacggaactcaccggcatcggcgccctgttgggcagtgaagacgacggttccaccaaaattaccggtatcgttgtgggagggccggctgacaaatccggagaattgaagctgaacgaccgcatcgttgccattgactccgacaactctggagaaatggtggatatcctgttcatgaagctggacaaagtggtggatatgatccgcggagccgaaaatacccagatgcgcctgaaagtagagccggcagacgcccctggacaggccaaaatcattacgctgacccgctccaaggtacctctgaaggatgaacttgccaaaggtgaaatcattgaacttaccggagctccggaaggcaggaaccgcattggcgtgctgagccttccctccttctacgcagacatggaaggcggagaccgccgctgtgccaaggatgtcaaaaaaatcctggaacggatgaacaaggaaaatgtggatggcctggtaattgacctgcgcagcaacggcggcggttccctggaggaagtgcgcctgatgacgggcttctttaccggaaacggccccgtggtgcaaatcaaggacacccgcggcaacgtggatatcaaatccgcccacaaccgccagaaactcttcaatggccccattgtggtgctcatcaataaactcagcgcatccgcctctgaaattctggctgcggcccttcaggattacggccgcgccgtgattgtgggggatgaatccaccttcgggaaggggtctgtgcagcagcctgtggacatcggccaatacctgcctttcttcgcggccagagaccgtgcgggcctgctgaaagtcactacccagaaattttaccgtgtggcgggcggctccacccagctcaaaggcgtggaaagcgatatccagcttcccaccgctacggcggcattcgaactgggagaagacattctggactacgcgatgccctatgaccagattacgccctgcaccaactacaaaaaggactcctccatcgcggccatgctgcccgtgctgaaagatgccagcgcgaagcgcgtggaaaaagaccgcgacctccagattgccagggaagatatcgccatgatgaaacagcgcatcaaggacaacaagctttccctgaacaagaaaatccgggaacaggaaaactccgccctggaagaacgccgcaaatccatcaacaaggaacgtaaaatccgcttcgcggaaatggccaaggaagacgctaccaaatacaaaatttaccgcctgacgctggacgacgtcaacgccaaggagctgcccctggcggatccggaaaaagacaatgaacaattcatgcacctggcggaagaccccacggcagaactggacgactccccggaatacccctccggccttgatccggaactccgcgaaggcatcaacatcgtccaggatatgctgaagctggaatcctccggaaaa

SEQ ID NO: 4 - protein, 745 aa, Unknown
  P9-02(10-37)-His-(38-748)
MNMHSFRWIRLTAFSALAAAAITSCASAHHHHHHATDFNQVGKQMSLLLQNFHFSRKEFSDELSTKFLETYLRKVDPNKIFFTQQDVDALKRKYGKELDDYLMSGQMMDAAQAMHALYRQRAMQRISYARDLLKKGGFTFDKDKSIERSRRKTAAWPKDEAEMQQVWKDMVEEQLLSEILRRETVARLAKEQNKPDPLANEKPAEEKLLMRYERIQRNIQETDLEDVAETLLSAVALTYDPHTDYMGARQVDRFKISMGTELTGIGALLGSEDDGSTKITGIVVGGPADKSGELKLNDRIVAIDSDNSGEMVDILFMKLDKVVDMIRGAENTQMRLKVEPADAPGQAKIITLTRSKVPLKDELAKGEIIELTGAPEGRNRIGVLSLPSFYADMEGGDRRCAKDVKKILERMNKENVDGLVIDLRSNGGGSLEEVRLMTGFFTGNGPVVQIKDTRGNVDIKSAHNRQKLFNGPIVVLINKLSASASEILAAALQDYGRAVIVGDESTFGKGSVQQPVDIGQYLPFFAARDRAGLLKVTTQKFYRVAGGSTQLKGVESDIQLPTATAAFELGEDILDYAMPYDQITPCTNYKKDSSIAAMLPVLKDASAKRVEKDRDLQIAREDIAMMKQRIKDNKLSLNKKIREQENSALEERRKSINKERKIRFAEMAKEDATKYKIYRLTLDDVNAKELPLADPEKDNEQFMHLAEDPTAELDDSPEYPSGLDPELREGINIVQDMLKLESSGK

SEQ ID NO: 5 - DNA, 55 bp, Unknown
  pET26b_P9-his_F
ttaactttaagaaggagatatacatatggaaaaaaacgcacccttttccgttatg

SEQ ID NO: 6 - DNA, 68 bp, Unknown
  pET26b_R
ttagcagccggatctcagtggtggtggtggtggtgctcgagttttccggaggattccagcttcagcat

SEQ ID NO: 7 - DNA, 60 bp, Unknown
  pET_P9_1_F
cctccggaaaactcgagcaccaccaccaccaccactgagatccggctgctaacaaagccc

SEQ ID NO: 8 - DNA, 50 bp, Unknown
  pET_P9_748-his_R
atgtatatctccttcttaaagttaaacaaaattatttctagaggggaatt

SEQ ID NO: 9 - DNA, 45 bp, Unknown
  pET_P9_delHis_F
agctggaatcctccggaaaatgagatccggctgctaacaaagccc

SEQ ID NO: 10 - DNA, 46 bp, Unknown
  pET_P9_delHis_R
ttgttagcagccggatctcattttccggaggattccagcttcagca

SEQ ID NO: 11 - DNA, 42 bp, Unknown
  pET_P9(His-38)_F
caccaccaccaccaccacgctacggacttcaaccaggtgggc

SEQ ID NO: 12 - DNA, 42 bp, Unknown
  pET_P9(His-38)_R
gtggtggtggtggtggtgcgcagaggcgcaggaagtaatggc

SEQ ID NO: 13 - DNA, 33 bp, Unknown
  P9_G45A_F
gacttcaaccaggtggccaagcaaatgtccctg

SEQ ID NO: 14 - DNA, 33 bp, Unknown
  P9_G45A_R
cagggacatttgcttggccacctggttgaagtc

SEQ ID NO: 15 - DNA, 33 bp, Unknown
  P9_G45V_F
gacttcaaccaggtggtcaagcaaatgtccctg

SEQ ID NO: 16 - DNA, 33 bp, Unknown
  P9_G45V_R
cagggacatttgcttgaccacctggttgaagtc

SEQ ID NO: 17 - DNA, 41 bp, Unknown
  P9_G45L_F
tacggacttcaaccaggtgctaaagcaaatgtccctgctgc

SEQ ID NO: 18 - DNA, 41 bp, Unknown
  P9_G45L_R
gcagcagggacatttgctttagcacctggttgaagtccgta

SEQ ID NO: 19 - DNA, 38 bp, Unknown
  P9_T263I_F
tcaaaatctccatgggtatagaactcaccggcatcggc

SEQ ID NO: 20 - DNA, 38 bp, Unknown
  P9_T263I_R
gccgatgccggtgagttctatacccatggagattttga

SEQ ID NO: 21 - DNA, 39 bp, Unknown
  P9_T263V_F
cgtttcaaaatctccatgggtgtggaactcaccggcatc

SEQ ID NO: 22 - DNA, 39 bp, Unknown
  P9_T263V_R
gatgccggtgagttccacacccatggagattttgaaacg

SEQ ID NO: 23 - DNA, 35 bp, Unknown
  P9_V423I_F
aaaatgtggatggcctgataattgacctgcgcagc

SEQ ID NO: 24 - DNA, 35 bp, Unknown
  P9_V423I_R
gctgcgcaggtcaattatcaggccatccacatttt

SEQ ID NO: 25 - DNA, 41 bp, Unknown
  P9_A492L_F
catccgcctctgaaattctgctagcggcccttcaggattac

SEQ ID NO: 26 - DNA, 41 bp, Unknown
  P9_A492L_R
gtaatcctgaagggccgctagcagaatttcagaggcggatg

SEQ ID NO: 27 - DNA, 31 bp, Unknown
  P9_A492V_F
cctctgaaattctggttgcggcccttcagga

SEQ ID NO: 28 - DNA, 31 bp, Unknown
  P9_A492V_R
tcctgaagggccgcaaccagaatttcagagg

SEQ ID NO: 29 - DNA, 29 bp, Unknown
  P9_L495I_F
ttctggctgcggccattcaggattacggc

SEQ ID NO: 30 - DNA, 29 bp, Unknown
  P9_L495I_R
gccgtaatcctgaatggccgcagccagaa

SEQ ID NO: 31 - DNA, 27 bp, Unknown
  P9_A501V_F
gattacggccgcgtcgtgattgtgggg

SEQ ID NO: 32 - DNA, 27 bp, Unknown
  P9_A501V_R
ccccacaatcacgacgcggccgtaatc

SEQ ID NO: 33 - DNA, 32 bp, Unknown
  P9_A501I_F
caggattacggccgcatcgtgattgtggggga

SEQ ID NO: 34 - DNA, 32 bp, Unknown
  P9_A501I_R
tcccccacaatcacgatgcggccgtaatcctg

SEQ ID NO: 35 - DNA, 29 bp, Unknown
  P9_G733A_F
ggaactccgcgaagccatcaacatcgtcc

SEQ ID NO: 36 - DNA, 29 bp, Unknown
  P9_G733A_R
ggacgatgttgatggcttcgcggagttcc

SEQ ID NO: 37 - DNA, 31 bp, Unknown
  P9_G733V_F
cggaactccgcgaagtcatcaacatcgtcca

SEQ ID NO: 38 - DNA, 31 bp, Unknown
  P9_G733V_R
tggacgatgttgatgacttcgcggagttccg

SEQ ID NO: 39 - DNA, 40 bp, Unknown
  P9_G369A_F
gaaggatgaacttgccaaagctgaaatcattgaacttacc

SEQ ID NO: 40 - DNA, 40 bp, Unknown
  P9_G369A_R
ggtaagttcaatgatttcagctttggcaagttcatccttc

SEQ ID NO: 41 - DNA, 45 bp, Unknown
  P9_K368Q_F
cctctgaaggatgaacttgcccagggtgaaatcattgaacttacc

SEQ ID NO: 42 - DNA, 45 bp, Unknown
  P9_K368Q_R
ggtaagttcaatgatttcaccctgggcaagttcatccttcagagg

SEQ ID NO: 43 - DNA, 35 bp, Unknown
  P9_C589S_F
atgaccagattacgcccagcaccaactacaaaaag

SEQ ID NO: 44 - DNA, 35 bp, Unknown
  P9_C589S_R
ctttttgtagttggtgctgggcgtaatctggtcat

SEQ ID NO: 45 - DNA, 41 bp, Unknown
  P9_C589T_F
ctatgaccagattacgcccaccaccaactacaaaaaggact

SEQ ID NO: 46 - DNA, 41 bp, Unknown
  P9_C589T_R
agtcctttttgtagttggtggtgggcgtaatctggtcatag

SEQ ID NO: 47 - DNA, 30 bp, Unknown
  P9_C34A_F
ccgccattacttccgccgcctctgcggcta

SEQ ID NO: 48 - DNA, 30 bp, Unknown
  P9_C34A_R
tagccgcagaggcggcggaagtaatggcgg

SEQ ID NO: 49 - DNA, 37 bp, Unknown
  P9_V78L_F
gaaacctacctgcgcaagttagaccccaacaaaatat

SEQ ID NO: 50 - DNA, 37 bp, Unknown
  P9_V78L_R
atattttgttggggtctaacttgcgcaggtaggtttc

SEQ ID NO: 51 - DNA, 30 bp, Unknown
  P9_A251P_F
gcatacggattacatgggtccgcgccaagt

SEQ ID NO: 52 - DNA, 30 bp, Unknown
  P9_A251P_R
acttggcgcggacccatgtaatccgtatgc

SEQ ID NO: 53 - DNA, 31 bp, Unknown
  P9_D307A_F
gcatcgttgccattgcctccgacaactctgg

SEQ ID NO: 54 - DNA, 31 bp, Unknown
  P9_D307A_R
ccagagttgtcggaggcaatggcaacgatgc

SEQ ID NO: 55 - DNA, 39 bp, Unknown
  P9_K324D_F
ctgttcatgaagctggacgatgtggtggatatgatccgc

SEQ ID NO: 56 - DNA, 39 bp, Unknown
  P9_K324D_R
gcggatcatatccaccacatcgtccagcttcatgaacag

SEQ ID NO: 57 - DNA, 34 bp, Unknown
  P9_K324N_F
cctgttcatgaagctggacaatgtggtggatatg

SEQ ID NO: 58 - DNA, 34 bp, Unknown
  P9_K324N_R
catatccaccacattgtccagcttcatgaacagg

SEQ ID NO: 59 - DNA, 36 bp, Unknown
  P9_M213Q_F
cccgcggaggaaaaactgcttcagcgttatgaacgc

SEQ ID NO: 60 - DNA, 36 bp, Unknown
  P9_M213Q_R
gcgttcataacgctgaagcagtttttcctccgcggg

SEQ ID NO: 61 - DNA, 25 bp, Unknown
  P9_R402S_F
ggcggagaccgcagctgtgccaagg

SEQ ID NO: 62 - DNA, 25 bp, Unknown
  P9_R402S_R
ccttggcacagctgcggtctccgcc

SEQ ID NO: 63 - DNA, 45 bp, Unknown
  P9_M414F_F
gtcaaaaaaatcctggaacggttcaacaaggaaaatgtggatggc

SEQ ID NO: 64 - DNA, 45 bp, Unknown; identical to SEQ ID NO: 63
  P9_M414F_R

SEQ ID NO: 65 - DNA, 42 bp, Unknown
  P9_M414I_F
caaaaaaatcctggaacggataaacaaggaaaatgtggatgg

SEQ ID NO: 66 - DNA, 42 bp, Unknown
  P9_M414I_R
ccatccacattttccttgtttatccgttccaggatttttttg

SEQ ID NO: 67 - DNA, 30 bp, Unknown
  P9_R438V_F
ccctggaggaagtggtcctgatgacgggct

SEQ ID NO: 68 - DNA, 30 bp, Unknown
  P9_R438V_R
agcccgtcatcaggaccacttcctccaggg

SEQ ID NO: 69 - DNA, 35 bp, Unknown
  P9_A465D_F
cgtggatatcaaatccgaccacaaccgccagaaac

SEQ ID NO: 70 - DNA, 35 bp, Unknown
  P9_A465D_R
gtttctggcggttgtggtcggatttgatatccacg

SEQ ID NO: 71 - DNA, 35 bp, Unknown
  P9_N467D_F
atatcaaatccgcccacgaccgccagaaactcttc

SEQ ID NO: 72 - DNA, 35 bp, Unknown
  P9_N467D_R
gaagagtttctggcggtcgtgggcggatttgatat

SEQ ID NO: 73 - DNA, 35 bp, Unknown
  P9_A534F_F
ttcttcgcggccagagaccgtttcggcctgctgaa

SEQ ID NO: 74 - DNA, 35 bp, Unknown
  P9_A534F_R
ttcagcaggccgaaacggtctctggccgcgaagaa

SEQ ID NO: 75 - DNA, 31 bp, Unknown
  P9_Y583F_F
gactacgcgatgccctttgaccagattacgc

SEQ ID NO: 76 - DNA, 31 bp, Unknown
  P9_Y583F_R
gcgtaatctggtcaaagggcatcgcgtagtc

SEQ ID NO: 77 - DNA, 39 bp, Unknown
  P9_A231F_F
acggatctggaagacgtattcgaaacactgctcagcgcc

SEQ ID NO: 78 - DNA, 39 bp, Unknown
  P9_A231F_R
ggcgctgagcagtgtttcgaatacgtcttccagatccgt

SEQ ID NO: 79 - DNA, 43 bp, Unknown
  P9_T263L_F
gtttcaaaatctccatgggtctagaactcaccggcatcggcgc

SEQ ID NO: 80 - DNA, 43 bp, Unknown
  P9_T263L_R
gcgccgatgccggtgagttctagacccatggagattttgaaac

SEQ ID NO: 81 - DNA, 28 bp, Unknown
  P9_C403T_F
cggagaccgccgcactgccaaggatgtc

SEQ ID NO: 82 - DNA, 28 bp, Unknown
  P9_C403T_R
gacatccttggcagtgcggcggtctccg

SEQ ID NO: 83 - DNA, 31 bp, Unknown
  P9_T445I_F
tgatgacgggcttctttatcggaaacggccc

SEQ ID NO: 84 - DNA, 31 bp, Unknown
  P9_T445I_R
gggccgtttccgataaagaagcccgtcatca

SEQ ID NO: 85 - DNA, 41 bp, Unknown
  P9_C589A_F
ctatgaccagattacgcccgccaccaactacaaaaaggact

SEQ ID NO: 86 - DNA, 41 bp, Unknown
  P9_C589A_R
agtcctttttgtagttggtggcgggcgtaatctggtcatag

SEQ ID NO: 87 - DNA, 28 bp, Unknown
  P9_C403A_F
cggagaccgccgcgctgccaaggatgtc

SEQ ID NO: 88 - DNA, 28 bp, Unknown
  P9_C403A_R
gacatccttggcagcgcggcggtctccg

SEQ ID NO: 89 - DNA, 34 bp, Unknown
  P9_K46A_F
cttcaaccaggtgggcgcgcaaatgtccctgctg

SEQ ID NO: 90 - DNA, 34 bp, Unknown
  P9_K46A_R
cagcagggacatttgcgcgcccacctggttgaag

SEQ ID NO: 91 - DNA, 49 bp, Unknown
  P9_R59A/K60A_F
gctccagaatttccacttctccgccgcagaattcagcgatgaactatcc

SEQ ID NO: 92 - DNA, 49 bp, Unknown
  P9_R59A/K60A_R
ggatagttcatcgctgaattctgcggcggagaagtggaaattctggagc

SEQ ID NO: 93 - DNA, 40 bp, Unknown
  P9_K82A_F
gcgcaaggtagaccccaacgcaatattcttcacccagcag

SEQ ID NO: 94 - DNA, 40 bp, Unknown
  P9_K82A_R
ctgctgggtgaagaatattgcgttggggtctaccttgcgc

SEQ ID NO: 95 - DNA, 52 bp, Unknown
  P9_K94A/R95A/K96A_F
ccagcaggacgtagacgccctcgcagcagcatacggtaaggagctggacgac

SEQ ID NO: 96 - DNA, 52 bp, Unknown
  P9_K94A/R95A/K96A_R
gtcgtccagctccttaccgtatgctgctgcgagggcgtctacgtcctgctgg

SEQ ID NO: 97 - DNA, 44 bp, Unknown
  P9_K368A_F
cctctgaaggatgaacttgccgcaggtgaaatcattgaacttac

SEQ ID NO: 98 - DNA, 44 bp, Unknown
  P9_K368A_R
gtaagttcaatgatttcacctgcggcaagttcatccttcagagg

SEQ ID NO: 99 - DNA, 37 bp, Unknown
  P9_K482A_F
gccccattgtggtgctcatcaatgcactcagcgcatc

SEQ ID NO: 100 - DNA, 37 bp, Unknown
  P9_K482A_R
gatgcgctgagtgcattgatgagcaccacaatggggc

SEQ ID NO: 101 - DNA, 32 bp, Unknown
  P9_R500A_F
cttcaggattacggcgccgccgtgattgtggg

SEQ ID NO: 102 - DNA, 32 bp, Unknown
  P9_R500A_R
cccacaatcacggcggcgccgtaatcctgaag

SEQ ID NO: 103 - DNA, 32 bp, Unknown
  P9_K512A_F
gaatccaccttcggggcggggtctgtgcagca

SEQ ID NO: 104 - DNA, 32 bp, Unknown
  P9_K512A_R
tgctgcacagaccccgccccgaaggtggattc

SEQ ID NO: 105 - DNA, 28 bp, Unknown
  P9_R531A_F
tttcttcgcggccgcagaccgtgcgggc

SEQ ID NO: 106 - DNA, 28 bp, Unknown
  P9_R531A_R
gcccgcacggtctgcggccgcgaagaaa

SEQ ID NO: 107 - DNA, 27 bp, Unknown
  P9_C34S_F
cgccattacttccagcgcctctgcgca

SEQ ID NO: 108 - DNA, 27 bp, Unknown
  P9_C34S_R
tgcgcagaggcgctggaagtaatggcg

SEQ ID NO: 109 - DNA, 44 bp, Unknown
  P9_S36H/A37H_F
cgccattacttcctgcgcccatcatcaccaccaccaccaccacg

SEQ ID NO: 110 - DNA, 44 bp, Unknown
  P9_S36H/A37H_R
cgtggtggtggtggtggtgatgatgggcgcaggaagtaatggcg

SEQ ID NO: 111 - DNA, 37 bp, Unknown
  P9_S486A_F
gctcatcaataaactcagcgcagccgcctctgaaatt

SEQ ID NO: 112 - DNA, 37 bp, Unknown
  P9_S486A_R
aatttcagaggcggctgcgctgagtttattgatgagc

SEQ ID NO: 113 - protein, 754 aa, Unknown
  P9-00(1-748-His)
MEKNAPFSVMNMHSFRWIRLTAFSALAAAAITSCASAATDFNQVGKQMSLLLQNFHFSRKEFSDELSTKFLETYLRKVDPNKIFFTQQDVDALKRKYGKELDDYLMSGQMMDAAQAMHALYRQRAMQRISYARDLLKKGGFTFDKDKSIERSRRKTAAWPKDEAEMQQVWKDMVEEQLLSEILRRETVARLAKEQNKPDPLANEKPAEEKLLMRYERIQRNIQETDLEDVAETLLSAVALTYDPHTDYMGARQVDRFKISMGTELTGIGALLGSEDDGSTKITGIVVGGPADKSGELKLNDRIVAIDSDNSGEMVDILFMKLDKVVDMIRGAENTQMRLKVEPADAPGQAKIITLTRSKVPLKDELAKGEIIELTGAPEGRNRIGVLSLPSFYADMEGGDRRCAKDVKKILERMNKENVDGLVIDLRSNGGGSLEEVRLMTGFFTGNGPVVQIKDTRGNVDIKSAHNRQKLFNGPIVVLINKLSASASEILAAALQDYGRAVIVGDESTFGKGSVQQPVDIGQYLPFFAARDRAGLLKVTTQKFYRVAGGSTQLKGVESDIQLPTATAAFELGEDILDYAMPYDQITPCTNYKKDSSIAAMLPVLKDASAKRVEKDRDLQIAREDIAMMKQRIKDNKLSLNKKIREQENSALEERRKSINKERKIRFAEMAKEDATKYKIYRLTLDDVNAKELPLADPEKDNEQFMHLAEDPTAELDDSPEYPSGLDPELREGINIVQDMLKLESSGKHHHHHH

SEQ ID NO: 114 - DNA, 39 bp, Unknown
  P9-2CA_Q43C_F
gcggctacggacttcaactgcgtgggcaagcaaatgtcc

SEQ ID NO: 115 - DNA, 39 bp, Unknown
  P9-2CA_Q43C_R
ggacatttgcttgcccacgcagttgaagtccgtagccgc

SEQ ID NO: 116 - DNA, 37 bp, Unknown
  P9-2CA_R59C_F
cagaatttccacttctcctgcaaagaattcagcgatg

SEQ ID NO: 117 - DNA, 37 bp, Unknown
  P9-2CA_R59C_R
catcgctgaattctttgcaggagaagtggaaattctg

SEQ ID NO: 118 - DNA, 39 bp, Unknown
  P9-2CA_R95C_F
gacgtagacgccctcaaatgcaaatacggtaaggagctg

SEQ ID NO: 119 - DNA, 39 bp, Unknown
  P9-2CA_R95C_R
cagctccttaccgtatttgcatttgagggcgtctacgtc

SEQ ID NO: 120 - DNA, 45 bp, Unknown
  P9-2CA_K99C_F
gccctcaaaagaaaatacggttgcgagctggacgactaccttatg

SEQ ID NO: 121 - DNA, 45 bp, Unknown
  P9-2CA-K99C-R
cataaggtagtcgtccagctcgcaaccgtattttcttttgagggc

SEQ ID NO: 122 - DNA, 30 bp, Unknown
  P9-2CA_S107C_F
ctggacgactaccttatgtgcggccagatg

SEQ ID NO: 123 - DNA, 30 bp, Unknown
  P9-2CA_S107C_R
catctggccgcacataaggtagtcgtccag

SEQ ID NO: 124 - DNA, 30 bp, Unknown
  P9-2CA_A119C_F
cccaggccatgcactgcctttaccgccagc

SEQ ID NO: 125 - DNA, 30 bp, Unknown
  P9-2CA_A119C_R
gctggcggtaaaggcagtgcatggcctggg

SEQ ID NO: 126 - DNA, 38 bp, Unknown
  P9-2CA_K138C_F
cctatgcgcgggatttgctgaaatgcggaggcttcacc

SEQ ID NO: 127 - DNA, 38 bp, Unknown
  P9-2CA_K138C_R
ggtgaagcctccgcatttcagcaaatcccgcgcatagg

SEQ ID NO: 128 - DNA, 40 bp, Unknown
  P9-2CA_T142C_F
gctgaaaaagggaggcttctgctttgacaaagacaagtct

SEQ ID NO: 129 - DNA, 40 bp, Unknown
  P9-2CA_T142C_R
agacttgtctttgtcaaagcagaagcctccctttttcagc

SEQ ID NO: 130 - DNA, 33 bp, Unknown
  P9-2CA_A158C_F
cgccgcaaaacagcctgctggcccaaggatgag

SEQ ID NO: 131 - DNA, 33 bp, Unknown
  P9-2CA_A158C_R
ctcatccttgggccagcaggctgttttgcggcg

SEQ ID NO: 132 - DNA, 33 bp, Unknown
  P9-2CA_K161C_F
acagccgcgtggccctgcgatgaggcggaaatg

SEQ ID NO: 133 - DNA, 33 bp, Unknown
  P9-2CA_K161C_R
catttccgcctcatcgcagggccacgcggctgt

SEQ ID NO: 134 - DNA, 37 bp, Unknown
  P9-2CA_A164C_F
cgtggcccaaggatgagtgcgaaatgcagcaggtctg

SEQ ID NO: 135 - DNA, 37 bp, Unknown
  P9-2CA_A164C_R
cagacctgctgcatttcgcactcatccttgggccacg

SEQ ID NO: 136 - DNA, 32 bp, Unknown
  P9-2CA_A189C_F
cctgcgccgtgaaaccgtatgccgcctggcca

SEQ ID NO: 137 - DNA, 32 bp, Unknown
  P9-2CA_A189C_R
tggccaggcggcatacggtttcacggcgcagg

SEQ ID NO: 138 - DNA, 33 bp, Unknown
  P9-2CA_K193C_F
gtagcgcgcctggcctgcgaacagaacaagccc

SEQ ID NO: 139 - DNA, 33 bp, Unknown
  P9-2CA_K193C_R
gggcttgttctgttcgcaggccaggcgcgctac

SEQ ID NO: 140 - DNA, 30 bp, Unknown
  P9-2CA_N203C_F
ccgatcccctggcctgtgaaaaacccgcgg

SEQ ID NO: 141 - DNA, 30 bp, Unknown
  P9-2CA_N203C_R
ccgcgggtttttcacaggccaggggatcgg

SEQ ID NO: 142 - DNA, 38 bp, Unknown
  P9-2CA_R220C_F
gcgttatgaacgcattcagtgcaatattcaggaaacgg

SEQ ID NO: 143 - DNA, 38 bp, Unknown
  P9-2CA_R220C_R
ccgtttcctgaatattgcactgaatgcgttcataacgc

SEQ ID NO: 144 - DNA, 41 bp, Unknown
  P9-2CA_K258C_F
gcgccaagtggaccgtttctgcatctccatgggtacggaac

SEQ ID NO: 145 - DNA, 41 bp, Unknown
  P9-2CA_K258C_R
gttccgtacccatggagatgcagaaacggtccacttggcgc

SEQ ID NO: 146 - DNA, 33 bp, Unknown
  P9-2CA_S311C_F
gccattgactccgacaactgtggagaaatggtg

SEQ ID NO: 147 - DNA, 33 bp, Unknown
  P9-2CA_S311C_R
caccatttctccacagttgtcggagtcaatggc

SEQ ID NO: 148 - DNA, 37 bp, Unknown
  P9-2CA_A332C_F
gtggtggatatgatccgcggatgcgaaaatacccaga

SEQ ID NO: 149 - DNA, 37 bp, Unknown
  P9-2CA_A332C_R
tctgggtattttcgcatccgcggatcatatccaccac

SEQ ID NO: 150 - DNA, 27 bp, Unknown
  P9-2CA_S358C_F
acgctgacccgctgcaaggtacctctg

SEQ ID NO: 151 - DNA, 27 bp, Unknown
  P9-2CA_S358C_R
cagaggtaccttgcagcgggtcagcgt

SEQ ID NO: 152 - DNA, 41 bp, Unknown
  P9-2CA_K363C_F
ccgctccaaggtacctctgtgcgatgaacttgccaaaggtg

SEQ ID NO: 153 - DNA, 41 bp, Unknown
  P9-2CA_K363C_R
cacctttggcaagttcatcgcacagaggtaccttggagcgg

SEQ ID NO: 154 - DNA, 37 bp, Unknown
  P9-2CA_E379C_F
aacttaccggagctccgtgcggcaggaaccgcattgg

SEQ ID NO: 155 - DNA, 37 bp, Unknown
  P9-2CA_E379C_R
ccaatgcggttcctgccgcacggagctccggtaagtt

SEQ ID NO: 156 - DNA, 38 bp, Unknown
  P9-2CA_K409C_F
gccaaggatgtcaaatgcatcctggaacggatgaacaa

SEQ ID NO: 157 - DNA, 38 bp, Unknown
  P9-2CA_K409C_R
ttgttcatccgttccaggatgcatttgacatccttggc

SEQ ID NO: 158 - DNA, 45 bp, Unknown
  P9-2CA_K416C_F
aaaatcctggaacggatgaactgcgaaaatgtggatggcctggta

SEQ ID NO: 159 - DNA, 45 bp, Unknown
  P9-2CA_K416C_R
taccaggccatccacattttcgcagttcatccgttccaggatttt

SEQ ID NO: 160 - DNA, 33 bp, Unknown
  P9-2CA_S464C_F
gcggcaacgtggatatcaaatgcgcccacaacc

SEQ ID NO: 161 - DNA, 33 bp, Unknown
  P9-2CA_S464C_R
ggttgtgggcgcatttgatatccacgttgccgc

SEQ ID NO: 162 - DNA, 35 bp, Unknown
  P9-2CA_R468C_F
tcaaatccgcccacaactgccagaaactcttcaat

SEQ ID NO: 163 - DNA, 35 bp, Unknown
  P9-2CA_R468C_R
attgaagagtttctggcagttgtgggcggatttga

SEQ ID NO: 164 - DNA, 39 bp, Unknown
  P9-2CA_Q523C_F
cagcctgtggacatcggctgctacctgcctttcttcgcg

SEQ ID NO: 165 - DNA, 39 bp, Unknown
  P9-2CA_Q523C_R
cgcgaagaaaggcaggtagcagccgatgtccacaggctg

SEQ ID NO: 166 - DNA, 30 bp, Unknown
  P9-2CA_A530C_F
tgcctttcttcgcgtgcagagaccgtgcgg

SEQ ID NO: 167 - DNA, 30 bp, Unknown
  P9-2CA_A530C_R
ccgcacggtctctgcacgcgaagaaaggca

SEQ ID NO: 168 - DNA, 40 bp, Unknown
  P9-2CA_Q562C_F
caaaggcgtggaaagcgatatctgccttcccaccgctacg

SEQ ID NO: 169 - DNA, 40 bp, Unknown
  P9-2CA_Q562C_R
cgtagcggtgggaaggcagatatcgctttccacgcctttg

SEQ ID NO: 170 - DNA, 40 bp, Unknown
  P9-2CA_D575C_F
ggcattcgaactgggagaatgcattctggactacgcgatg

SEQ ID NO: 171 - DNA, 40 bp, Unknown
  P9-2CA_D575C_R
catcgcgtagtccagaatgcattctcccagttcgaatgcc

SEQ ID NO: 172 - DNA, 39 bp, Unknown
  P9-2CA_Q585C_F
tacgcgatgccctatgactgcattacgcccgccaccaac

SEQ ID NO: 173 - DNA, 39 bp, Unknown
  P9-2CA_Q585C_R
gttggtggcgggcgtaatgcagtcatagggcatcgcgta

SEQ ID NO: 174 - DNA, 38 bp, Unknown
  P9-2CA_T590C_F
gaccagattacgcccgcctgcaactacaaaaaggactc

SEQ ID NO: 175 - DNA, 38 bp, Unknown
  P9-2CA_T590C_R
gagtcctttttgtagttgcaggcgggcgtaatctggtc

SEQ ID NO: 176 - DNA, 34 bp, Unknown
  P9-2CA_S596C_F
ccaactacaaaaaggactgctccatcgcggccat

SEQ ID NO: 177 - DNA, 34 bp, Unknown
  P9-2CA_S596C_R
atggccgcgatggagcagtcctttttgtagttgg

SEQ ID NO: 178 - DNA, 39 bp, Unknown
  P9-2CA_A610C_F
gtgctgaaagatgccagctgcaagcgcgtggaaaaagac

SEQ ID NO: 179 - DNA, 39 bp, Unknown
  P9-2CA_A610C_R
gtctttttccacgcgcttgcagctggcatctttcagcac

SEQ ID NO: 180 - DNA, 40 bp, Unknown
  P9-2CA_A627C_F
gattgccagggaagatatctgcatgatgaaacagcgcatc

SEQ ID NO: 181 - DNA, 40 bp, Unknown
  P9-2CA_A627C_R
gatgcgctgtttcatcatgcagatatcttccctggcaatc

SEQ ID NO: 182 - DNA, 45 bp, Unknown
  P9-2CA_K634C_F
gccatgatgaaacagcgcatctgcgacaacaagctttccctgaac

SEQ ID NO: 183 - DNA, 45 bp, Unknown
  P9-2CA_K634C_R
gttcagggaaagcttgttgtcgcagatgcgctgtttcatcatggc

SEQ ID NO: 184 - DNA, 34 bp, Unknown
  P9-2CA_A651C_F
ggaacaggaaaactcctgcctggaagaacgccgc

SEQ ID NO: 185 - DNA, 34 bp, Unknown
  P9-2CA_A651C_R
gcggcgttcttccaggcaggagttttcctgttcc

SEQ ID NO: 186 - DNA, 34 bp, Unknown
  P9-2CA_S658C_F
ggaagaacgccgcaaatgcatcaacaaggaacgt

SEQ ID NO: 187 - DNA, 34 bp, Unknown
  P9-2CA_S658C_R
acgttccttgttgatgcatttgcggcgttcttcc

SEQ ID NO: 188 - DNA, 42 bp, Unknown
  P9-2CA_K700C_F
gcccctggcggatccggaatgcgacaatgaacaattcatgca

SEQ ID NO: 189 - DNA, 42 bp, Unknown
  P9-2CA_K700C_R
tgcatgaattgttcattgtcgcattccggatccgccaggggc

SEQ ID NO: 190 - DNA, 39 bp, Unknown
  P9-2CA_E710C_F
caattcatgcacctggcgtgcgaccccacggcagaactg

SEQ ID NO: 191 - DNA, 39 bp, Unknown
  P9-2CA_E710C_R
cagttctgccgtggggtcgcacgccaggtgcatgaattg

SEQ ID NO: 192 - DNA, 35 bp, Unknown
  P9-2CA_S745C_F
caggatatgctgaagctggaatgctccggaaaatg

SEQ ID NO: 193 - DNA, 35 bp, Unknown
  P9-2CA_S745C_R
cattttccggagcattccagcttcagcatatcctg